European Patent Application EP 4 257 144 A1, published October 11, 2023. Title: A pharmaceutical composition for preventing or treating bone disorders, comprising Trigonal glucagon/GLP-1/GIP receptor agonist or a conjugate thereof. Applicant: HANMI PHARM. CO., LTD. The sequence listing filed with the application follows.

SEQUENCE LISTING (134 sequences)

SEQ ID NO: 1 - protein, 30 aa, Artificial Sequence
  Trigonal agonist
  MISC_FEATURE (2): Xaa is 2-aminoisobutyric acid (Aib)
HXQGTFTSDVSSYLDGQAAKEFIAWLVKGC

SEQ ID NO: 2 - protein, 30 aa, Artificial Sequence
  Trigonal agonist
  MISC_FEATURE (2): Xaa is 2-aminoisobutyric acid (Aib)
HXQGTFTSDVSSYLDGQAQKEFIAWLVKGC

SEQ ID NO: 3 - protein, 41 aa, Artificial Sequence
  Trigonal agonist
  MISC_FEATURE (2): Xaa is 2-aminoisobutyric acid (Aib)
HXQGTFTSDVSSYLLGQAAKQFIAWLVKGGGPSSGAPPPSC

SEQ ID NO: 4 - protein, 30 aa, Artificial Sequence
  Trigonal agonist
  MISC_FEATURE (2): Xaa is 2-aminoisobutyric acid (Aib)
HXQGTFTSDVSSYLLGQQQKEFIAWLVKGC

SEQ ID NO: 5 - protein, 41 aa, Artificial Sequence
  Trigonal agonist
  MISC_FEATURE (2): Xaa is 2-aminoisobutyric acid (Aib)
HXQGTFTSDVSSYLLGQQQKEFIAWLVKGGGPSSGAPPPSC

SEQ ID NO: 6 - protein, 30 aa, Artificial Sequence
  Trigonal agonist
  MISC_FEATURE (2): Xaa is 2-aminoisobutyric acid (Aib)
HXQGTFTSDVSSYLDGQAAKEFVAWLLKGC

SEQ ID NO: 7 - protein, 30 aa, Artificial Sequence
  Trigonal agonist
  MISC_FEATURE (2): Xaa is 2-aminoisobutyric acid (Aib)
HXQGTFTSDVSKYLDGQAAKEFVAWLLKGC

SEQ ID NO: 8 - protein, 30 aa, Artificial Sequence
  Trigonal agonist
  MISC_FEATURE (2): Xaa is 2-aminoisobutyric acid (Aib)
HXQGTFTSDVSKYLDGQAAQEFVAWLLKGC

SEQ ID NO: 9 - protein, 30 aa, Artificial Sequence
  Trigonal agonist
  MISC_FEATURE (2): Xaa is 2-aminoisobutyric acid (Aib)
HXQGTFTSDVSKYLDGQAAQEFVAWLLAGC

SEQ ID NO: 10 - protein, 41 aa, Artificial Sequence
  Trigonal agonist
  MISC_FEATURE (2): Xaa is 2-aminoisobutyric acid (Aib)
HXQGTFTSDVSKYLDGQAAQEFVAWLLAGGGPSSGAPPPSC

SEQ ID NO: 11 - protein, 41 aa, Artificial Sequence
  Trigonal agonist
  MISC_FEATURE (1): Xaa is 4-imidazoacetyl (CA)
XGEGTFTSDLSKYLDSRRQQLFVQWLKAGGPSSGAPPPSHG

SEQ ID NO: 12 - protein, 41 aa, Artificial Sequence
  Trigonal agonist
  MISC_FEATURE (1): Xaa is 4-imidazoacetyl (CA)
XGEGTFISDLSKYMDEQAVQLFVEWLMAGGPSSGAPPPSHG

SEQ ID NO: 13 - protein, 41 aa, Artificial Sequence
  Trigonal agonist
  MISC_FEATURE (1): Xaa is 4-imidazoacetyl (CA)
XGEGTFISDYSIQLDEIAVQDFVEWLLAQKPSSGAPPPSHG

SEQ ID NO: 14 - protein, 41 aa, Artificial Sequence
  Trigonal agonist
  MISC_FEATURE (1): Xaa is 4-imidazoacetyl (CA)
XGQGTFTSDYSIQLDEIAVRDFVEWLKNGGPSSGAPPPSHG

SEQ ID NO: 15 - protein, 41 aa, Artificial Sequence
  Trigonal agonist
  MISC_FEATURE (1): Xaa is 4-imidazoacetyl (CA)
XGQGTFTSDLSKQMDEEAVRLFIEWLKNGGPSSGAPPPSHG

SEQ ID NO: 16 - protein, 41 aa, Artificial Sequence
  Trigonal agonist
  MISC_FEATURE (1): Xaa is 4-imidazoacetyl (CA)
XGQGTFTSDLSKQMDSEAQQLFIEWLKNGGPSSGAPPPSHG

SEQ ID NO: 17 - protein, 41 aa, Artificial Sequence
  Trigonal agonist
  MISC_FEATURE (1): Xaa is 4-imidazoacetyl (CA)
XGQGTFTSDLSKQMDEERAREFIEWLLAQKPSSGAPPPSHG

SEQ ID NO: 18 - protein, 41 aa, Artificial Sequence
  Trigonal agonist
  MISC_FEATURE (1): Xaa is 4-imidazoacetyl (CA)
XGQGTFTSDLSKQMDSERAREFIEWLKNTGPSSGAPPPSHG

SEQ ID NO: 19 - protein, 41 aa, Artificial Sequence
  Trigonal agonist
  MISC_FEATURE (1): Xaa is 4-imidazoacetyl (CA)
XGQGTFTSDLSIQYDSEHQRDFIEWLKDTGPSSGAPPPSHG

SEQ ID NO: 20 - protein, 41 aa, Artificial Sequence
  Trigonal agonist
  MISC_FEATURE (1): Xaa is 4-imidazoacetyl (CA)
XGQGTFTSDLSIQYEEEAQQDFVEWLKDTGPSSGAPPPSHG

SEQ ID NO: 21 - protein, 39 aa, Artificial Sequence
  Trigonal agonist
  MISC_FEATURE (2): Xaa is 2-aminoisobutyric acid (Aib)
  MISC_FEATURE (16)..(20): amino acids at positions 16 and 20 form a ring
YXQGTFTSDYSKYLDECRAKEFVQWLLDHHPSSGQPPPS

SEQ ID NO: 22 - protein, 39 aa, Artificial Sequence
  Trigonal agonist
  MISC_FEATURE (2): Xaa is 2-aminoisobutyric acid (Aib)
  MISC_FEATURE (16)..(20): amino acids at positions 16 and 20 form a ring
YXQGTFTSDYSKCLDEKRAKEFVQWLLDHHPSSGQPPPS

SEQ ID NO: 23 - protein, 41 aa, Artificial Sequence
  Trigonal agonist
  MISC_FEATURE (2): Xaa is 2-aminoisobutyric acid (Aib)
  MISC_FEATURE (16)..(20): amino acids at positions 16 and 20 form a ring
YXQGTFTSDYSKYLDECRAKEFVQWLLAQKGKKNDWKHNIT

SEQ ID NO: 24 - protein, 39 aa, Artificial Sequence
  Trigonal agonist
  MISC_FEATURE (2): Xaa is 2-aminoisobutyric acid (Aib)
  MISC_FEATURE (16)..(20): amino acids at positions 16 and 20 form a ring
YXQGTFTSDYSKYLDECRAKEFVQWLKNGGPSSGAPPPS

SEQ ID NO: 25 - protein, 39 aa, Artificial Sequence
  Trigonal agonist
  MISC_FEATURE (2): Xaa is 2-aminoisobutyric acid (Aib)
HXQGTFTSDCSKYLDERAAQDFVQWLLDGGPSSGAPPPS

SEQ ID NO: 26 - protein, 39 aa, Artificial Sequence
  Trigonal agonist
  MISC_FEATURE (2): Xaa is 2-aminoisobutyric acid (Aib)
HXQGTFTSDCSKYLDSRAAQDFVQWLLDGGPSSGAPPPS

SEQ ID NO: 27 - protein, 40 aa, Artificial Sequence
  Trigonal agonist
  MISC_FEATURE (2): Xaa is 2-aminoisobutyric acid (Aib)
HXQGTFTSDYSKYLDERACQDFVQWLLDQGGPSSGAPPPS

SEQ ID NO: 28 - protein, 41 aa, Artificial Sequence
  Trigonal agonist
  MISC_FEATURE (2): Xaa is 2-aminoisobutyric acid (Aib)
HXQGTFTSDYSKYLDEKRAQEFVCWLLAQKGKKNDWKHNIT

SEQ ID NO: 29 - protein, 30 aa, Artificial Sequence
  Trigonal agonist
  MISC_FEATURE (2): Xaa is 2-aminoisobutyric acid (Aib)
  MISC_FEATURE (16)..(20): amino acids at positions 16 and 20 form a ring
HXQGTFTSDYSKYLDEKAAKEFVQWLLNTC

SEQ ID NO: 30 - protein, 30 aa, Artificial Sequence
  Trigonal agonist
  MISC_FEATURE (2): Xaa is 2-aminoisobutyric acid (Aib)
  MISC_FEATURE (16)..(20): amino acids at positions 16 and 20 form a ring
HXQGTFTSDYSKYLDEKAQKEFVQWLLDTC

SEQ ID NO: 31 - protein, 29 aa, Artificial Sequence
  Trigonal agonist
  MISC_FEATURE (2): Xaa is 2-aminoisobutyric acid (Aib)
  MISC_FEATURE (16)..(20): amino acids at positions 16 and 20 form a ring
HXQGTFTSDYSKYLDEKACKEFVQWLLAQ

SEQ ID NO: 32 - protein, 39 aa, Artificial Sequence
  Trigonal agonist
  MISC_FEATURE (2): Xaa is 2-aminoisobutyric acid (Aib)
  MISC_FEATURE (16)..(20): amino acids at positions 16 and 20 form a ring
HXQGTFTSDYSKYLDEKACKDFVQWLLDGGPSSGAPPPS

SEQ ID NO: 33 - protein, 31 aa, Artificial Sequence
  Trigonal agonist
  MISC_FEATURE (2): Xaa is 2-aminoisobutyric acid (Aib)
  MISC_FEATURE (16)..(20): amino acids at positions 16 and 20 form a ring
HXQGTFTSDYSIAMDEIHQKDFVNWLLAQKC

SEQ ID NO: 34 - protein, 31 aa, Artificial Sequence
  Trigonal agonist
  MISC_FEATURE (2): Xaa is 2-aminoisobutyric acid (Aib)
  MISC_FEATURE (16)..(20): amino acids at positions 16 and 20 form a ring
HXQGTFTSDYSKYLDEKRQKEFVNWLLAQKC

SEQ ID NO: 35 - protein, 31 aa, Artificial Sequence
  Trigonal agonist
  MISC_FEATURE (2): Xaa is 2-aminoisobutyric acid (Aib)
  MISC_FEATURE (16)..(20): amino acids at positions 16 and 20 form a ring
HXQGTFTSDYSIAMDEIHQKDFVNWLLNTKC

SEQ ID NO: 36 - protein, 40 aa, Artificial Sequence
  Trigonal agonist
  MISC_FEATURE (2): Xaa is 2-aminoisobutyric acid (Aib)
  MISC_FEATURE (16)..(20): amino acids at positions 16 and 20 form a ring
HXQGTFTSDYSKYLCEKRQKEFVQWLLNGGPSSGAPPPSG

SEQ ID NO: 37 - protein, 40 aa, Artificial Sequence
  Trigonal agonist
  MISC_FEATURE (2): Xaa is 2-aminoisobutyric acid (Aib)
  MISC_FEATURE (16)..(20): amino acids at positions 16 and 20 form a ring
HXQGTFTSDYSKYLDECRQKEFVQWLLNGGPSSGAPPPSG

SEQ ID NO: 38 - protein, 40 aa, Artificial Sequence
  Trigonal agonist
  MISC_FEATURE (1): Xaa is 4-imidazoacetyl (CA)
  MISC_FEATURE (2): Xaa is 2-aminoisobutyric acid (Aib)
XXQGTFTSDKSSYLDERAAQDFVQWLLDGGPSSGAPPPSS

SEQ ID NO: 39 - protein, 40 aa, Artificial Sequence
  Trigonal agonist
  MISC_FEATURE (2): Xaa is 2-aminoisobutyric acid (Aib)
HXQGTFTSDYSKYLDGQHAQCFVAWLLAGGGPSSGAPPPS

SEQ ID NO: 40 - protein, 39 aa, Artificial Sequence
  Trigonal agonist
  MISC_FEATURE (2): Xaa is 2-aminoisobutyric acid (Aib)
HXQGTFTSDKSKYLDERACQDFVQWLLDGGPSSGAPPPS

SEQ ID NO: 41 - protein, 39 aa, Artificial Sequence
  Trigonal agonist
  MISC_FEATURE (2): Xaa is 2-aminoisobutyric acid (Aib)
HXQGTFTSDKSKYLDECAAQDFVQWLLDGGPSSGAPPPS

SEQ ID NO: 42 - protein, 40 aa, Artificial Sequence
  Trigonal agonist
  MISC_FEATURE (2): Xaa is 2-aminoisobutyric acid (Aib)
  MISC_FEATURE (16)..(20): amino acids at positions 16 and 20 form a ring
YXQGTFTSDYSKYLDEKRAKEFVQWLLDHHPSSGQPPPSC

SEQ ID NO: 43 - protein, 39 aa, Artificial Sequence
  Trigonal agonist
  MISC_FEATURE (2): Xaa is 2-aminoisobutyric acid (Aib)
  MISC_FEATURE (16)..(20): amino acids at positions 16 and 20 form a ring
YXQGTFTSDYSKYLDEKRAKEFVQWLLDHHCSSGQPPPS

SEQ ID NO: 44 - protein, 39 aa, Artificial Sequence
  Trigonal agonist
HGQGTFTSDCSKQLDGQAAQEFVAWLLAGGPSSGAPPPS

SEQ ID NO: 45 - protein, 39 aa, Artificial Sequence
  Trigonal agonist
HGQGTFTSDCSKYMDGQAAQDFVAWLLAGGPSSGAPPPS

SEQ ID NO: 46 - protein, 39 aa, Artificial Sequence
  Trigonal agonist
HGQGTFTSDCSKYLDEQHAQEFVAWLLAGGPSSGAPPPS

SEQ ID NO: 47 - protein, 39 aa, Artificial Sequence
  Trigonal agonist
HGQGTFTSDCSKYLDGQRAQEFVAWLLAGGPSSGAPPPS

SEQ ID NO: 48 - protein, 39 aa, Artificial Sequence
  Trigonal agonist
HGQGTFTSDCSKYLDGQRAQDFVNWLLAGGPSSGAPPPS

SEQ ID NO: 49 - protein, 30 aa, Artificial Sequence
  Trigonal agonist
  MISC_FEATURE (1): Xaa is 4-imidazoacetyl (CA)
  MISC_FEATURE (2): Xaa is 2-aminoisobutyric acid (Aib)
  MISC_FEATURE (16)..(20): amino acids at positions 16 and 20 form a ring
XXQGTFTSDYSICMDEIHQKDFVNWLLNTK

SEQ ID NO: 50 - protein, 40 aa, Artificial Sequence
  Trigonal agonist
  MISC_FEATURE (2): Xaa is 2-aminoisobutyric acid (Aib)
  MISC_FEATURE (16)..(20): amino acids at positions 16 and 20 form a ring
HXQGTFTSDYSKYLDEKRAKEFVQWLLDHHPSSGQPPPSC

SEQ ID NO: 51 - protein, 30 aa, Artificial Sequence
  Trigonal agonist
  MISC_FEATURE (2): Xaa is 2-aminoisobutyric acid (Aib)
  MISC_FEATURE (16)..(20): amino acids at positions 16 and 20 form a ring
HXQGTFTSDYSKYLDEKRQKEFVQWLLNTC

SEQ ID NO: 52 - protein, 30 aa, Artificial Sequence
  Trigonal agonist
  MISC_FEATURE (2): Xaa is 2-aminoisobutyric acid (Aib)
  MISC_FEATURE (16)..(20): amino acids at positions 16 and 20 form a ring
HXQGTFTSDYSKYLDEKRQKEFVQWLLDTC

SEQ ID NO: 53 - protein, 30 aa, Artificial Sequence
  Trigonal agonist
  MISC_FEATURE (2): Xaa is 2-aminoisobutyric acid (Aib)
  MISC_FEATURE (16)..(20): amino acids at positions 16 and 20 form a ring
HXEGTFTSDYSIAMDEIHQKDFVNWLLAQC

SEQ ID NO: 54 - protein, 30 aa, Artificial Sequence
  Trigonal agonist
  MISC_FEATURE (2): Xaa is 2-aminoisobutyric acid (Aib)
  MISC_FEATURE (16)..(20): amino acids at positions 16 and 20 form a ring
HXEGTFTSDYSIAMDEIHQKDFVDWLLAEC

SEQ ID NO: 55 - protein, 30 aa, Artificial Sequence
  Trigonal agonist
  MISC_FEATURE (2): Xaa is 2-aminoisobutyric acid (Aib)
  MISC_FEATURE (16)..(20): amino acids at positions 16 and 20 form a ring
HXQGTFTSDYSIAMDEIHQKDFVNWLLAQC

SEQ ID NO: 56 - protein, 30 aa, Artificial Sequence
  Trigonal agonist
  MISC_FEATURE (2): Xaa is 2-aminoisobutyric acid (Aib)
  MISC_FEATURE (16)..(20): amino acids at positions 16 and 20 form a ring
HXQGTFTSDYSKYLDEKRQKEFVNWLLAQC

SEQ ID NO: 57 - protein, 30 aa, Artificial Sequence
  Trigonal agonist
  MISC_FEATURE (2): Xaa is 2-aminoisobutyric acid (Aib)
  MISC_FEATURE (16)..(20): amino acids at positions 16 and 20 form a ring
HXQGTFTSDYSIAMDEIHQKDFVNWLLNTC

SEQ ID NO: 58 - protein, 31 aa, Artificial Sequence
  Trigonal agonist
  MISC_FEATURE (2): Xaa is 2-aminoisobutyric acid (Aib)
  MISC_FEATURE (16)..(20): amino acids at positions 16 and 20 form a ring
HXQGTFTSDYSKYLDEKRQKEFVQWLLNTKC

SEQ ID NO: 59 - protein, 30 aa, Artificial Sequence
  Trigonal agonist
  MISC_FEATURE (1): Xaa is 4-imidazoacetyl (CA)
  MISC_FEATURE (2): Xaa is 2-aminoisobutyric acid (Aib)
  MISC_FEATURE (16)..(20): amino acids at positions 16 and 20 form a ring
XXQGTFTSDYSICMDEKHQKDFVNWLLNTK

SEQ ID NO: 60 - protein, 30 aa, Artificial Sequence
  Trigonal agonist
  MISC_FEATURE (1): Xaa is 4-imidazoacetyl (CA)
  MISC_FEATURE (2): Xaa is 2-aminoisobutyric acid (Aib)
  MISC_FEATURE (16)..(20): amino acids at positions 16 and 20 form a ring
XXQGTFTSDYSIAMDEKHCKDFVNWLLNTK

SEQ ID NO: 61 - protein, 30 aa, Artificial Sequence
  Trigonal agonist
  MISC_FEATURE (1): Xaa is 4-imidazoacetyl (CA)
  MISC_FEATURE (2): Xaa is 2-aminoisobutyric acid (Aib)
  MISC_FEATURE (16)..(20): amino acids at positions 16 and 20 form a ring
XXQGTFTSDYSIAMDEIACKDFVNWLLNTK

SEQ ID NO: 62 - protein, 39 aa, Artificial Sequence
  Trigonal agonist
  MISC_FEATURE (1): Xaa is 4-imidazoacetyl (CA)
  MISC_FEATURE (2): Xaa is 2-aminoisobutyric acid (Aib)
XXQGTFTSDKSKYLDERAAQDFVQWLLDGGPSSGAPPPS

SEQ ID NO: 63 - protein, 39 aa, Artificial Sequence
  Trigonal agonist
  MISC_FEATURE (1): Xaa is 4-imidazoacetyl (CA)
  MISC_FEATURE (2): Xaa is 2-aminoisobutyric acid (Aib)
XXQGTFTSDCSKYLDERAAQDFVQWLLDGGPSSGAPPPS

SEQ ID NO: 64 - protein, 39 aa, Artificial Sequence
  Trigonal agonist
  MISC_FEATURE (2): Xaa is 2-aminoisobutyric acid (Aib)
  MISC_FEATURE (16)..(20): amino acids at positions 16 and 20 form a ring
YXQGTFTSDYSKYLDECAAKEFVQWLLDHHPSSGQPPPS

SEQ ID NO: 65 - protein, 39 aa, Artificial Sequence
  Trigonal agonist
  MISC_FEATURE (2): Xaa is 2-aminoisobutyric acid (Aib)
  MISC_FEATURE (16)..(20): amino acids at positions 16 and 20 form a ring
HXQGTFTSDYSKCLDEKRAKEFVQWLLDHHPSSGQPPPS

SEQ ID NO: 66 - protein, 39 aa, Artificial Sequence
  Trigonal agonist
  MISC_FEATURE (2): Xaa is 2-aminoisobutyric acid (Aib)
  MISC_FEATURE (16)..(20): amino acids at positions 16 and 20 form a ring
YXQGTFTSDYSKYLDECRAKDFVQWLLDHHPSSGQPPPS

SEQ ID NO: 67 - protein, 39 aa, Artificial Sequence
  Trigonal agonist
  MISC_FEATURE (2): Xaa is 2-aminoisobutyric acid (Aib)
  MISC_FEATURE (16)..(20): amino acids at positions 16 and 20 form a ring
YXQGTFTSDYSKYLDECAAKDFVQWLLDHHPSSGQPPPS

SEQ ID NO: 68 - protein, 39 aa, Artificial Sequence
  Trigonal agonist
  MISC_FEATURE (2): Xaa is 2-aminoisobutyric acid (Aib)
  MISC_FEATURE (16)..(20): amino acids at positions 16 and 20 form a ring
YXQGTFTSDYSKCLDEKAAKEFVQWLLDHHPSSGQPPPS

SEQ ID NO: 69 - protein, 39 aa, Artificial Sequence
  Trigonal agonist
  MISC_FEATURE (2): Xaa is 2-aminoisobutyric acid (Aib)
  MISC_FEATURE (16)..(20): amino acids at positions 16 and 20 form a ring
YXQGTFTSDYSKCLDERAAKEFVQWLLDHHPSSGQPPPS

SEQ ID NO: 70 - protein, 39 aa, Artificial Sequence
  Trigonal agonist
  MISC_FEATURE (2): Xaa is 2-aminoisobutyric acid (Aib)
  MISC_FEATURE (16)..(20): amino acids at positions 16 and 20 form a ring
YXQGTFTSDYSKCLDEKRAKDFVQWLLDHHPSSGQPPPS

SEQ ID NO: 71 - protein, 39 aa, Artificial Sequence
  Trigonal agonist
  MISC_FEATURE (2): Xaa is 2-aminoisobutyric acid (Aib)
  MISC_FEATURE (16)..(20): amino acids at positions 16 and 20 form a ring
YXQGTFTSDYSKYLDERACKDFVQWLLDHHPSSGQPPPS

SEQ ID NO: 72 - protein, 39 aa, Artificial Sequence
  Trigonal agonist
  MISC_FEATURE (2): Xaa is 2-aminoisobutyric acid (Aib)
  MISC_FEATURE (16)..(20): amino acids at positions 16 and 20 form a ring
YXQGTFTSDCSKYLDERAAKDFVQWLLDHHPSSGQPPPS

SEQ ID NO: 73 - protein, 39 aa, Artificial Sequence
  Trigonal agonist
  MISC_FEATURE (1): Xaa is 4-imidazoacetyl (CA)
  MISC_FEATURE (2): Xaa is 2-aminoisobutyric acid (Aib)
  MISC_FEATURE (16)..(20): amino acids at positions 16 and 20 form a ring
XXQGTFTSDYSKYLDECRAKEFVQWLLDHHPSSGQPPPS

SEQ ID NO: 74 - protein, 39 aa, Artificial Sequence
  Trigonal agonist
  MISC_FEATURE (1): Xaa is 4-imidazoacetyl (CA)
  MISC_FEATURE (2): Xaa is 2-aminoisobutyric acid (Aib)
  MISC_FEATURE (16)..(20): amino acids at positions 16 and 20 form a ring
XXQGTFTSDYSKCLDEKRAKEFVQWLLDHHPSSGQPPPS

SEQ ID NO: 75 - protein, 40 aa, Artificial Sequence
  Trigonal agonist
  MISC_FEATURE (2): Xaa is 2-aminoisobutyric acid (Aib)
  MISC_FEATURE (16)..(20): amino acids at positions 16 and 20 form a ring
YXQGTFTSDYSKYLDEKAAKEFVQWLLDHHPSSGQPPPSC

SEQ ID NO: 76 - protein, 40 aa, Artificial Sequence
  Trigonal agonist
  MISC_FEATURE (2): Xaa is 2-aminoisobutyric acid (Aib)
  MISC_FEATURE (16)..(20): amino acids at positions 16 and 20 form a ring
YXQGTFTSDYSKYLDEKRAKDFVQWLLDHHPSSGQPPPSC

SEQ ID NO: 77 - protein, 40 aa, Artificial Sequence
  Trigonal agonist
  MISC_FEATURE (2): Xaa is 2-aminoisobutyric acid (Aib)
  MISC_FEATURE (16)..(20): amino acids at positions 16 and 20 form a ring
YXQGTFTSDYSKYLDEKAAKDFVQWLLDHHPSSGQPPPSC

SEQ ID NO: 78 - protein, 31 aa, Artificial Sequence
  Trigonal agonist
  MISC_FEATURE (2): Xaa is 2-aminoisobutyric acid (Aib)
  MISC_FEATURE (16)..(20): amino acids at positions 16 and 20 form a ring
HXQGTFTSDYSKYLDEKRQKEFVQWLLDTKC

SEQ ID NO: 79 - protein, 31 aa, Artificial Sequence
  Trigonal agonist
  MISC_FEATURE (2): Xaa is 2-aminoisobutyric acid (Aib)
  MISC_FEATURE (16)..(20): amino acids at positions 16 and 20 form a ring
HXEGTFTSDYSIAMDEIHQKDFVNWLLAQKC

SEQ ID NO: 80 - protein, 31 aa, Artificial Sequence
  Trigonal agonist
  MISC_FEATURE (2): Xaa is 2-aminoisobutyric acid (Aib)
  MISC_FEATURE (16)..(20): amino acids at positions 16 and 20 form a ring
HXEGTFTSDYSIAMDEIHQKDFVDWLLAEKC

SEQ ID NO: 81 - protein, 30 aa, Artificial Sequence
  Trigonal agonist
  MISC_FEATURE (1): Xaa is 4-imidazoacetyl (CA)
  MISC_FEATURE (2): Xaa is 2-aminoisobutyric acid (Aib)
  MISC_FEATURE (16)..(20): amino acids at positions 16 and 20 form a ring
XXQGTFTSDYSKYLDEKRQKEFVQWLLNTC

SEQ ID NO: 82 - protein, 30 aa, Artificial Sequence
  Trigonal agonist
  MISC_FEATURE (1): Xaa is 4-imidazoacetyl (CA)
  MISC_FEATURE (2): Xaa is 2-aminoisobutyric acid (Aib)
  MISC_FEATURE (16)..(20): amino acids at positions 16 and 20 form a ring
XXQGTFTSDYSKYLDEKRQKEFVQWLLDTC

SEQ ID NO: 83 - protein, 30 aa, Artificial Sequence
  Trigonal agonist
  MISC_FEATURE (1): Xaa is 4-imidazoacetyl (CA)
  MISC_FEATURE (2): Xaa is 2-aminoisobutyric acid (Aib)
  MISC_FEATURE (16)..(20): amino acids at positions 16 and 20 form a ring
XXEGTFTSDYSIAMDEIHQKDFVNWLLAQC

SEQ ID NO: 84 - protein, 30 aa, Artificial Sequence
  Trigonal agonist
  MISC_FEATURE (1): Xaa is 4-imidazoacetyl (CA)
  MISC_FEATURE (2): Xaa is 2-aminoisobutyric acid (Aib)
  MISC_FEATURE (16)..(20): amino acids at positions 16 and 20 form a ring
XXEGTFTSDYSIAMDEIHQKDFVDWLLAEC

SEQ ID NO: 85 - protein, 30 aa, Artificial Sequence
  Trigonal agonist
  MISC_FEATURE (1): Xaa is 4-imidazoacetyl (CA)
  MISC_FEATURE (2): Xaa is 2-aminoisobutyric acid (Aib)
  MISC_FEATURE (16)..(20): amino acids at positions 16 and 20 form a ring
XXQGTFTSDYSIAMDEIHQKDFVNWLLAQC

SEQ ID NO: 86 - protein, 30 aa, Artificial Sequence
  Trigonal agonist
  MISC_FEATURE (1): Xaa is 4-imidazoacetyl (CA)
  MISC_FEATURE (2): Xaa is 2-aminoisobutyric acid (Aib)
  MISC_FEATURE (16)..(20): amino acids at positions 16 and 20 form a ring
XXQGTFTSDYSKYLDEKRQKEFVNWLLAQC

SEQ ID NO: 87 - protein, 30 aa, Artificial Sequence
  Trigonal agonist
  MISC_FEATURE (1): Xaa is 4-imidazoacetyl (CA)
  MISC_FEATURE (2): Xaa is 2-aminoisobutyric acid (Aib)
  MISC_FEATURE (16)..(20): amino acids at positions 16 and 20 form a ring
XXQGTFTSDYSIAMDEIHQKDFVNWLLNTC

SEQ ID NO: 88 - protein, 31 aa, Artificial Sequence
  Trigonal agonist
  MISC_FEATURE (1): Xaa is 4-imidazoacetyl (CA)
  MISC_FEATURE (2): Xaa is 2-aminoisobutyric acid (Aib)
  MISC_FEATURE (16)..(20): amino acids at positions 16 and 20 form a ring
XXQGTFTSDYSKYLDEKRQKEFVQWLLNTKC

SEQ ID NO: 89 - protein, 31 aa, Artificial Sequence
  Trigonal agonist
  MISC_FEATURE (1): Xaa is 4-imidazoacetyl (CA)
  MISC_FEATURE (2): Xaa is 2-aminoisobutyric acid (Aib)
  MISC_FEATURE (16)..(20): amino acids at positions 16 and 20 form a ring
XXQGTFTSDYSKYLDEKRQKEFVQWLLDTKC

SEQ ID NO: 90 - protein, 31 aa, Artificial Sequence
  Trigonal agonist
  MISC_FEATURE (1): Xaa is 4-imidazoacetyl (CA)
  MISC_FEATURE (2): Xaa is 2-aminoisobutyric acid (Aib)
  MISC_FEATURE (16)..(20): amino acids at positions 16 and 20 form a ring
XXEGTFTSDYSIAMDEIHQKDFVNWLLAQKC

SEQ ID NO: 91 - protein, 31 aa, Artificial Sequence
  Trigonal agonist
  MISC_FEATURE (1): Xaa is 4-imidazoacetyl (CA)
  MISC_FEATURE (2): Xaa is 2-aminoisobutyric acid (Aib)
  MISC_FEATURE (16)..(20): amino acids at positions 16 and 20 form a ring
XXEGTFTSDYSIAMDEIHQKDFVDWLLAEKC

SEQ ID NO: 92 - protein, 31 aa, Artificial Sequence
  Trigonal agonist
  MISC_FEATURE (1): Xaa is 4-imidazoacetyl (CA)
  MISC_FEATURE (2): Xaa is 2-aminoisobutyric acid (Aib)
  MISC_FEATURE (16)..(20): amino acids at positions 16 and 20 form a ring
XXQGTFTSDYSIAMDEIHQKDFVNWLLAQKC

SEQ ID NO: 93 - protein, 31 aa, Artificial Sequence
  Trigonal agonist
  MISC_FEATURE (1): Xaa is 4-imidazoacetyl (CA)
  MISC_FEATURE (2): Xaa is 2-aminoisobutyric acid (Aib)
  MISC_FEATURE (16)..(20): amino acids at positions 16 and 20 form a ring
XXQGTFTSDYSKYLDEKRQKEFVNWLLAQKC

SEQ ID NO: 94 - protein, 31 aa, Artificial Sequence
  Trigonal agonist
  MISC_FEATURE (1): Xaa is 4-imidazoacetyl (CA)
  MISC_FEATURE (2): Xaa is 2-aminoisobutyric acid (Aib)
  MISC_FEATURE (16)..(20): amino acids at positions 16 and 20 form a ring
XXQGTFTSDYSIAMDEIHQKDFVNWLLNTKC

SEQ ID NO: 95 - protein, 39 aa, Artificial Sequence
  Trigonal agonist
  MISC_FEATURE (2): Xaa is 2-aminoisobutyric acid (Aib)
  MISC_FEATURE (16)..(20): amino acids at positions 16 and 20 form a ring
YXQGTFTSDYSKYLDEKRAKEFVQWLLCHHPSSGQPPPS

SEQ ID NO: 96 - protein, 39 aa, Artificial Sequence
  Trigonal agonist
  MISC_FEATURE (2): Xaa is 2-aminoisobutyric acid (Aib)
  MISC_FEATURE (16)..(20): amino acids at positions 16 and 20 form a ring
YXQGTFTSDYSKYLDEKRAKEFVQWLLDHCPSSGQPPPS

SEQ ID NO: 97 - protein, 39 aa, Artificial Sequence
  Trigonal agonist
  MISC_FEATURE (2): Xaa is 2-aminoisobutyric acid (Aib)
  MISC_FEATURE (16)..(20): amino acids at positions 16 and 20 form a ring
YXQGTFTSDYSKYLDEKRAKEFVQWLLDCHPSSGQPPPS

SEQ ID NO: 98 - protein, 40 aa, Artificial Sequence
  Trigonal agonist
  MISC_FEATURE (2): Xaa is 2-aminoisobutyric acid (Aib)
  MISC_FEATURE (16)..(20): amino acids at positions 16 and 20 form a ring
YXQGTFTSDYSKALDEKAAKEFVNWLLDHHPSSGQPPPSC

SEQ ID NO: 99 - protein, 40 aa, Artificial Sequence
  Trigonal agonist
  MISC_FEATURE (2): Xaa is 2-aminoisobutyric acid (Aib)
  MISC_FEATURE (16)..(20): amino acids at positions 16 and 20 form a ring
YXQGTFTSDYSKALDEKAAKDFVNWLLDHHPSSGQPPPSC

SEQ ID NO: 100 - protein, 40 aa, Artificial Sequence
  Trigonal agonist
  MISC_FEATURE (2): Xaa is 2-aminoisobutyric acid (Aib)
  MISC_FEATURE (16)..(20): amino acids at positions 16 and 20 form a ring
YXQGTFTSDYSKALDEKAAKEFVQWLLDQHPSSGQPPPSC

SEQ ID NO: 101 - protein, 40 aa, Artificial Sequence
  Trigonal agonist
  MISC_FEATURE (2): Xaa is 2-aminoisobutyric acid (Aib)
  MISC_FEATURE (16)..(20): amino acids at positions 16 and 20 form a ring
YXQGTFTSDYSKALDEKAAKEFVNWLLDQHPSSGQPPPSC

SEQ ID NO: 102 - protein, 40 aa, Artificial Sequence
  Trigonal agonist
  MISC_FEATURE (2): Xaa is 2-aminoisobutyric acid (Aib)
  MISC_FEATURE (16)..(20): amino acids at positions 16 and 20 form a ring
YXQGTFTSDYSKALDEKAAKDFVNWLLDQHPSSGQPPPSC

SEQ ID NO: 103 - protein, 12 aa, HOMO SAPIENS
ESKYGPPCPSCP

SEQ ID NO: 104 - protein, 11 aa, Artificial Sequence
  Variant of hinge region
ESKYGPPPSCP

SEQ ID NO: 105 - protein, 11 aa, Artificial Sequence
  Variant of hinge region
ESKYGPPCPSP

SEQ ID NO: 106 - protein, 10 aa, Artificial Sequence
  Variant of hinge region
ESKYGPPCPS

SEQ ID NO: 107 - protein, 10 aa, Artificial Sequence
  Variant of hinge region
ESKYGPPCPP

SEQ ID NO: 108 - protein, 8 aa, Artificial Sequence
  Variant of hinge region
KYGPPCPS

SEQ ID NO: 109 - protein, 8 aa, Artificial Sequence
  Variant of hinge region
ESKYGPPC

SEQ ID NO: 110 - protein, 7 aa, Artificial Sequence
  Variant of hinge region
EKYGPPC

SEQ ID NO: 111 - protein, 6 aa, Artificial Sequence
  Variant of hinge region
ESPSCP

SEQ ID NO: 112 - protein, 5 aa, Artificial Sequence
  Variant of hinge region
EPSCP

SEQ ID NO: 113 - protein, 4 aa, Artificial Sequence
  Variant of hinge region
PSCP

SEQ ID NO: 114 - protein, 10 aa, Artificial Sequence
  Variant of hinge region
ESKYGPPSCP

SEQ ID NO: 115 - protein, 9 aa, Artificial Sequence
  Variant of hinge region
KYGPPPSCP

SEQ ID NO: 116 - protein, 9 aa, Artificial Sequence
  Variant of hinge region
ESKYGPSCP

SEQ ID NO: 117 - protein, 8 aa, Artificial Sequence
  Variant of hinge region
ESKYGPPC

SEQ ID NO: 118 - protein, 7 aa, Artificial Sequence
  Variant of hinge region
KYGPPCP

SEQ ID NO: 119 - protein, 7 aa, Artificial Sequence
  Variant of hinge region
ESKPSCP

SEQ ID NO: 120 - protein, 6 aa, Artificial Sequence
  Variant of hinge region
ESPSCP

SEQ ID NO: 121 - protein, 4 aa, Artificial Sequence
  Variant of hinge region
EPSC

SEQ ID NO: 122 - protein, 3 aa, Artificial Sequence
  Variant of hinge region
SCP

SEQ ID NO: 123 - protein, 221 aa, homo sapiens
PSCPAPEFLGGPSVFLFPPKPKDTLMISRTPEVTCVVVDVSQEDPEVQFNWYVDGVEVHNAKTKPREEQFNSTYRVVSVLTVLHQDWLNGKEYKCKVSNKGLPSSIEKTISKAKGQPREPQVYTLPPSQEEMTKNQVSLTCLVKGFYPSDIAVEWESNGQPENNYKTTPPVLDSDGSFFLYSRLTVDKSRWQEGNVFSCSVMHEALHNHYTQKSLSLSLGK

SEQ ID NO: 124 - DNA, 21 bp, Artificial Sequence
  Forward primer of RUNX2
gccctcatccttcactccaag

SEQ ID NO: 125 - DNA, 21 bp, Artificial Sequence
  Reverse primer of RUNX2
ggtcagtcagtgcctttcctc

SEQ ID NO: 126 - DNA, 20 bp, Artificial Sequence
  Forward primer of OCN
gagggcaataaggtagtgaa

SEQ ID NO: 127 - DNA, 19 bp, Artificial Sequence
  Reverse primer of OCN
catagatgcgtttgtaggc

SEQ ID NO: 128 - DNA, 20 bp, Artificial Sequence
  Forward primer of ALP
ccagcaggtttctctcttgg

SEQ ID NO: 129 - DNA, 20 bp, Artificial Sequence
  Reverse primer of ALP
ggaatgttccatggaggttg

SEQ ID NO: 130 - DNA, 20 bp, Artificial Sequence
  Forward primer of ColA1
agagcatgaccgatggattc

SEQ ID NO: 131 - DNA, 20 bp, Artificial Sequence
  Reverse primer of ColA1
ccttcttgaggttgccagtc

SEQ ID NO: 132 - DNA, 19 bp, Artificial Sequence
  Forward primer of GAPDH
gtcgtggatctgacgtgcc

SEQ ID NO: 133 - DNA, 19 bp, Artificial Sequence
  Reverse primer of GAPDH
tgcctgcttcaccaccttc

SEQ ID NO: 134 - protein, 442 aa, Homo sapiens
  MISC_FEATURE (1)..(442): Amino acids at position 1 to 442 form Human Immunoglobulin G4 Fc Fragment (homodimer)
  MISC_FEATURE (1)..(221): Amino acids at position 1 to 221 form one monomer
  MISC_FEATURE (222)..(442): Amino acids at position 222 to 442 form one monomer
  DISULFID (3)..(224): Amino acids at position 3 and position 224 form an inter-disulfide bond
  DISULFID (35)..(95): Amino acids at position 35 and position 95 form an intra-chain disulfide bond
  DISULFID (141)..(199): Amino acids at position 141 and position 199 form an intra-chain disulfide bond
  DISULFID (256)..(316): Amino acids at position 256 and position 316 form an intra-chain disulfide bond
  DISULFID (362)..(420): Amino acids at position 362 and position 420 form an intra-chain disulfide bond
PSCPAPEFLGGPSVFLFPPKPKDTLMISRTPEVTCVVVDVSQEDPEVQFNWYVDGVEVHNAKTKPREEQFNSTYRVVSVLTVLHQDWLNGKEYKCKVSNKGLPSSIEKTISKAKGQPREPQVYTLPPSQEEMTKNQVSLTCLVKGFYPSDIAVEWESNGQPENNYKTTPPVLDSDGSFFLYSRLTVDKSRWQEGNVFSCSVMHEALHNHYTQKSLSLSLGKPSCPAPEFLGGPSVFLFPPKPKDTLMISRTPEVTCVVVDVSQEDPEVQFNWYVDGVEVHNAKTKPREEQFNSTYRVVSVLTVLHQDWLNGKEYKCKVSNKGLPSSIEKTISKAKGQPREPQVYTLPPSQEEMTKNQVSLTCLVKGFYPSDIAVEWESNGQPENNYKTTPPVLDSDGSFFLYSRLTVDKSRWQEGNVFSCSVMHEALHNHYTQKSLSLSLGK